European Patent Specification EP 3 713 964 B1, published January 17, 2024. Title: mRNA DISPLAY ANTIBODY LIBRARY AND METHODS. Applicant: NantBio, Inc. The sequence listing filed with the application follows.

SEQUENCE LISTING (45 sequences)

SEQ ID NO: 1 - DNA, 58 bp, Artificial Sequence
  Artificial Sequence for VH CDR1
ggcttaggtctcatttcrvtagttacgctatgcattgggcgagacgaggtctgaacgg

SEQ ID NO: 2 - DNA, 58 bp, Artificial Sequence
  Artificial Sequence for VH CDR1
ggcttaggtctcatttctctrvktacgctatgcattgggcgagacgaggtctgaacgg

SEQ ID NO: 3 - DNA, 58 bp, Artificial Sequence
  Artificial Sequence for VH CDR1
ggcttaggtctcatttctctagttackkgatgcattgggcgagacgaggtctgaacgg

SEQ ID NO: 4 - DNA, 58 bp, Artificial Sequence
  Artificial Sequence for VH CDR1
ggcttaggtctcatttctctagttacwmtatgcattgggcgagacgaggtctgaacgg

SEQ ID NO: 5 - DNA, 58 bp, Artificial Sequence
  Artificial Sequence for VH CDR1
ggcttaggtctcatttctctagttacgctatgavttgggcgagacgaggtctgaacgg

SEQ ID NO: 6 - DNA, 54 bp, Artificial Sequence
  Artificial Sequence for VH CDR2-n
ggcttaggtctcgttcathcattagtggtagtggacgagacgaggtctgaacgg

SEQ ID NO: 7 - DNA, 54 bp, Artificial Sequence
  Artificial Sequence for VH CDR2-n
ggcttaggtctcgttcavktattagtggtagtggacgagacgaggtctgaacgg

SEQ ID NO: 8 - DNA, 54 bp, Artificial Sequence
  Artificial Sequence for VH CDR2-n
ggcttaggtctcgttcagctattyggggtagtggacgagacgaggtctgaacgg

SEQ ID NO: 9 - DNA, 54 bp, Artificial Sequence
  Artificial Sequence for VH CDR2-n
ggcttaggtctcgttcagctattdatggtaatggacgagacgaggtctgaacgg

SEQ ID NO: 10 - DNA, 54 bp, Artificial Sequence
  Artificial Sequence for VH CDR2-n
ggcttaggtctcgttcagctattagtwmtagtggacgagacgaggtctgaacgg

SEQ ID NO: 11 - DNA, 54 bp, Artificial Sequence
  Artificial Sequence for VH CDR2-n
ggcttaggtctcgttcagctattagtkggagtggacgagacgaggtctgaacgg

SEQ ID NO: 12 - DNA, 54 bp, Artificial Sequence
  Artificial Sequence for VH CDR2-n
ggcttaggtctcgttcagctattagtggtrrtggacgagacgaggtctgaacgg

SEQ ID NO: 13 - DNA, 52 bp, Artificial Sequence
  Artificial Sequence for VH CDR2-c
ggcttaggtctcgtggarvkagtacttactacgcgagacgaggtctgaacgg

SEQ ID NO: 14 - DNA, 52 bp, Artificial Sequence
  Artificial Sequence for VH CDR2-c
  misc_feature (21)..(21): n is a, c, g, or t
ggcttaggtctcgtggaggtnatacttactacgcgagacgaggtctgaacgg

SEQ ID NO: 15 - DNA, 52 bp, Artificial Sequence
  Artificial Sequence for VH CDR2-c
ggcttaggtctcgtggaggtrvaacttactacgcgagacgaggtctgaacgg

SEQ ID NO: 16 - DNA, 52 bp, Artificial Sequence
  Artificial Sequence for VH CDR2-c
ggcttaggtctcgtggaggtagtactvrttacgcgagacgaggtctgaacgg

SEQ ID NO: 17 - DNA, 53 bp, Artificial Sequence
  Artificial Sequence for VH CDR3
  misc_feature (24)..(25): n is a, c, g, or t
  misc_feature (27)..(27): n is a, c, g, or t
ggcttaggtctctccgtgrtckcnnkngstttcgcgagacgaggtctgaacgg

SEQ ID NO: 18 - DNA, 58 bp, Artificial Sequence
  Artificial Sequence for VL CDR3
ggcttaggtctctgcagdsgdmtrvtdsgccttwcacttcgagacgaggtctgaacgg

SEQ ID NO: 19 - DNA, 58 bp, Artificial Sequence
  Artificial Sequence for VL CDR3
ggcttaggtctctgcagbwtdmtrvtdsgccttwcacttcgagacgaggtctgaacgg

SEQ ID NO: 20 - DNA, 58 bp, Artificial Sequence
  Artificial Sequence for VL CDR3
  misc_feature (27)..(27): n is a, c, g, or t
ggcttaggtctctgcagdsgdmtrvtnwtccttwcacttcgagacgaggtctgaacgg

SEQ ID NO: 21 - DNA, 58 bp, Artificial Sequence
  Artificial Sequence for VL CDR3
  misc_feature (27)..(27): n is a, c, g, or t
ggcttaggtctctgcagbwtdmtrvtnwtccttwcacttcgagacgaggtctgaacgg

SEQ ID NO: 22 - DNA, 58 bp, Artificial Sequence
  Artificial Sequence for VL CDR3
ggcttaggtctctgcagdsgdmtrvtdsgcctykgacttcgagacgaggtctgaacgg

SEQ ID NO: 23 - DNA, 58 bp, Artificial Sequence
  Artificial Sequence for VL CDR3
ggcttaggtctctgcagbwtdmtrvtdsgcctykgacttcgagacgaggtctgaacgg

SEQ ID NO: 24 - DNA, 58 bp, Artificial Sequence
  Artificial Sequence for VL CDR3
  misc_feature (27)..(27): n is a, c, g, or t
ggcttaggtctctgcagdsgdmtrvtnwtcctykgacttcgagacgaggtctgaacgg

SEQ ID NO: 25 - DNA, 58 bp, Artificial Sequence
  Artificial Sequence for VL CDR3
  misc_feature (27)..(27): n is a, c, g, or t
ggcttaggtctctgcagbwtdmtrvtnwtcctykgacttcgagacgaggtctgaacgg

SEQ ID NO: 26 - protein, 6 aa, Artificial Sequence
  Clone 801 CDRH1
NSYAMH

SEQ ID NO: 27 - protein, 10 aa, Artificial Sequence
  Clone 801 CDRH2
AISGNGGSTR

SEQ ID NO: 28 - protein, 8 aa, Artificial Sequence
  Clone 801 CDRH3
DRFRKVHG

SEQ ID NO: 29 - protein, 6 aa, Artificial Sequence
  Clone 801 CDRL3
DATFPL

SEQ ID NO: 30 - protein, 6 aa, Artificial Sequence
  Clone 802 CDRH1
GSYAMH

SEQ ID NO: 31 - protein, 10 aa, Artificial Sequence
  Clone 802 CDRH2
AISGSGGSTR

SEQ ID NO: 32 - protein, 8 aa, Artificial Sequence
  Clone 802 CDRH3
DLYRRVHG

SEQ ID NO: 33 - protein, 6 aa, Artificial Sequence
  Clone 802 CDRL3
DYGFPL

SEQ ID NO: 34 - protein, 6 aa, Artificial Sequence
  Clone 905 CDRH1
SSYLMH

SEQ ID NO: 35 - protein, 10 aa, Artificial Sequence
  Clone 905 CDRH2
VISGSGGSTR

SEQ ID NO: 36 - protein, 8 aa, Artificial Sequence
  Clone 905 CDRH3
DLYRRVAG

SEQ ID NO: 37 - protein, 6 aa, Artificial Sequence
  Clone 905 CDRL3
DYALPL

SEQ ID NO: 38 - protein, 6 aa, Artificial Sequence
  Clone 906 CDRH1
SNYAMH

SEQ ID NO: 39 - protein, 10 aa, Artificial Sequence
  Clone 906 CDRH2
AISGNGGSTH

SEQ ID NO: 40 - protein, 8 aa, Artificial Sequence
  Clone 906 CDRH3
DRFRRVYG

SEQ ID NO: 41 - protein, 6 aa, Artificial Sequence
  Clone 906 CDRL3
DYTFPL

SEQ ID NO: 42 - protein, 6 aa, Artificial Sequence
  Clone 817 CDRH1
SSYAMH

SEQ ID NO: 43 - protein, 10 aa, Artificial Sequence
  Clone 817 CDRH2
AISGSGGSTR

SEQ ID NO: 44 - protein, 7 aa, Artificial Sequence
  Clone 817 CDRH3
GRWSKWG

SEQ ID NO: 45 - protein, 6 aa, Artificial Sequence
  Clone 817 CDRL3
TDNFPY